European Patent Application EP 4 253 411 A1, published October 4, 2023. Title: MOLECULE SPECIFICALLY BINDING TO CLDN18.2. Applicant: SANYOU BIOPHARMACEUTICALS CO., LTD. The sequence listing filed with the application follows.

SEQUENCE LISTING (48 sequences)

SEQ ID NO: 1 - protein, 8 aa, Artificial Sequence
  CDR1
GSIFSINV

SEQ ID NO: 2 - protein, 7 aa, Artificial Sequence
  CDR2
ISTGGTT

SEQ ID NO: 3 - protein, 17 aa, Artificial Sequence
  CDR3
NADLATATSWPVRYLEV

SEQ ID NO: 4 - protein, 8 aa, Artificial Sequence
  CDR1
GSFFRIVA

SEQ ID NO: 5 - protein, 7 aa, Artificial Sequence
  CDR2
ITRGGST

SEQ ID NO: 6 - protein, 14 aa, Artificial Sequence
  CDR3
NVRVEVPFMQPNDY

SEQ ID NO: 7 - protein, 8 aa, Artificial Sequence
  CDR1
GRTFSNYA

SEQ ID NO: 8 - protein, 8 aa, Artificial Sequence
  CDR2
ITWSGGST

SEQ ID NO: 9 - protein, 15 aa, Artificial Sequence
  CDR3
AGGFFATSYSGNYGY

SEQ ID NO: 10 - protein, 123 aa, Artificial Sequence
  NA4-S VHH
EVQVVESGGGLVQPGGSLRLSCAASGSIFSINVMGWYRQAPGKQRELVAGISTGGTTRYADSAKGRFTISRDNAKNTVYLQMNSLKPEDTAVYYCNADLATATSWPVRYLEVWGQGTLVTVSA

SEQ ID NO: 11 - protein, 120 aa, Artificial Sequence
  NA7-S VHH
EVQVQESGGGLVQPGGSLRLSCAASGSFFRIVAMGWYRQAPGSQRELVATITRGGSTYYADSMKGRSTISRDNAKNTVYLQMNSLKPEDTAVYYCNVRVEVPFMQPNDYWGHGTQVTVSS

SEQ ID NO: 12 - protein, 122 aa, Artificial Sequence
  NA8-S VHH
EVQVQESGGGLVQAGGSLRLSCAASGRTFSNYAVGWFRQAPGKEREFVAAITWSGGSTNYADSVKGRFTISRDNAKNTAWLQMNSLKPEDTAVYYCAGGFFATSYSGNYGYWGQGTQVTVSS

SEQ ID NO: 13 - protein, 123 aa, Artificial Sequence
  NA4-S-H7 VHH
EVQLVESGGGLVQPGGSLRLSCAASGSIFSINVMGWYRQAPGKQRELVAGISTGGTTRYADSVKGRFTISRDNAKNTLYLQMNSLRAEDTAVYYCNADLATATSWPVRYLEVWGQGTLVTVSS

SEQ ID NO: 14 - protein, 120 aa, Artificial Sequence
  NA7-S-H2 VHH
EVQLVESGGGLVQPGGSLRLSCAASGSFFRIVAMGWYRQAPGKGRELVATITRGGSTYYADSMKGRSTISRDNAKNTVYLQMNSLKPEDTAVYYCNVRVEVPFMQPNDYWGQGTLVTVSS

SEQ ID NO: 15 - protein, 122 aa, Artificial Sequence
  NA8-S-H9 VHH
EVQLVESGGGLVQPGGSLRLSCAASGRTFSNYAVGWFRQAPGKGLEFVAAITWSGGSTNYADSVKGRFTISRDNAKNTLYLQMNSLRAEDTAVYYCAGGFFATSYSGNYGYWGQGTLVTVSS

SEQ ID NO: 16 - protein, 261 aa, Homo sapiens
MAVTACQGLGFVVSLIGIAGIIAATCMDQWSTQDLYNNPVTAVFNYQGLWRSCVRESSGFTECRGYFTLLGLPAMLQAVRALMIVGIVLGAIGLLVSIFALKCIRIGSMEDSAKANMTLTSGIMFIVSGLCAIAGVSVFANMLVTNFWMSTANMYTGMGGMVQTVQTRYTFGAALFVGWVAGGLTLIGGVMMCIACRGLAPEETNYKAVSYHASGHSVAYKPGGFKASTGFGSNTKNKKIYDGGARTEDEVQSYPSKHDYV

SEQ ID NO: 17 - protein, 261 aa, Homo sapiens
MSTTTCQVVAFLLSILGLAGCIAATGMDMWSTQDLYDNPVTSVFQYEGLWRSCVRQSSGFTECRPYFTILGLPAMLQAVRALMIVGIVLGAIGLLVSIFALKCIRIGSMEDSAKANMTLTSGIMFIVSGLCAIAGVSVFANMLVTNFWMSTANMYTGMGGMVQTVQTRYTFGAALFVGWVAGGLTLIGGVMMCIACRGLAPEETNYKAVSYHASGHSVAYKPGGFKASTGFGSNTKNKKIYDGGARTEDEVQSYPSKHDYV

SEQ ID NO: 18 - protein, 264 aa, Mus musculus
MSVTACQGLGFVVSLIGFAGIIAATCMDQWSTQDLYNNPVTAVFNYQGLWRSCVRESSGFTECRGYFTLLGLPAMLQAVRALMIVGIVLGVIGILVSIFALKCIRIGSMDDSAKAKMTLTSGILFIISGICAIIGVSVFANMLVTNFWMSTANMYSGMGGMGGMVQTVQTRYTFGAALFVGWVAGGLTLIGGVMMCIACRGLTPDDSNFKAVSYHASGQNVAYRPGGFKASTGFGSNTRNKKIYDGGARTEDDEQSHPTKYDYV

SEQ ID NO: 19 - protein, 264 aa, Mus musculus
MATTTCQVVGLLLSLLGLAGCIAATGMDMWSTQDLYDNPVTAVFQYEGLWRSCVQQSSGFTECRPYFTILGLPAMLQAVRALMIVGIVLGVIGILVSIFALKCIRIGSMDDSAKAKMTLTSGILFIISGICAIIGVSVFANMLVTNFWMSTANMYSGMGGMGGMVQTVQTRYTFGAALFVGWVAGGLTLIGGVMMCIACRGLTPDDSNFKAVSYHASGQNVAYRPGGFKASTGFGSNTRNKKIYDGGARTEDDEQSHPTKYDYV

SEQ ID NO: 20 - protein, 129 aa, Artificial Sequence
  Extracellular domain 1 of human CLDN18.2
METDTLLLWVLLLWVPGSTGDAAQPARRARRTKLGTELGSTPVWWNSADGRMDQWSTQDLYNNPVTAVFNYQGLWRSCVRESSGFTECRGYFTLLGLPAMLQAVRAAIQHSGGRSRRARTKTHLRRGSE

SEQ ID NO: 21 - protein, 232 aa, Artificial Sequence
  Human IgG1 Fc
EPKSCDKTHTCPPCPAPELLGGPSVFLFPPKPKDTLMISRTPEVTCVVVDVSHEDPEVKFNWYVDGVEVHNAKTKPREEQYNSTYRVVSVLTVLHQDWLNGKEYKCKVSNKALPAPIEKTISKAKGQPREPQVYTLPPSRDELTKNQVSLTCLVKGFYPSDIAVEWESNGQPENNYKTTPPVLDSDGSFFLYSKLTVDKSRWQQGNVFSCSVMHEALHNHYTQKSLSLSPGK

SEQ ID NO: 22 - protein, 14 aa, Artificial Sequence
  Intracellular antibody recognition segment of CLDN18
GFKASTGFGSNTKN

SEQ ID NO: 23 - protein, 120 aa, Artificial Sequence
  NA7S-H2-418 VHH
EVQLVESGGGLVQPGGSLRLSCAASGSFFRIVAMEWYRQAPGKGRELVATITRGGSTYYADSMKGRSTISRDNAKNTVYLQMNSLKPEDTAVYYCNVRVEVPFMQPNDYWGQGTLVTVSS

SEQ ID NO: 24 - protein, 120 aa, Artificial Sequence
  NA7S-H2-420 VHH
EVQLVESGGGLVQPGGSLRLSCAASGSFFRIVMYGWYRQAPGKGRELVATITRGGSTYYADSMKGRSTISRDNAKNTVYLQMNSLKPEDTAVYYCNVRVEVPFMQPNDYWGQGTLVTVSS

SEQ ID NO: 25 - protein, 120 aa, Artificial Sequence
  NA7S-H2-20 VHH
EVQLVESGGGLVQPGGSLRLSCAASGSFFRIVAMGWYRQAPGKGRELVATITRGGSTYYADSMKGRSTISRDNAKNTVYLQMNSLKPEDTAVYYCNVRVEVPFMAPNDYWGQGTLVTVSS

SEQ ID NO: 26 - protein, 120 aa, Artificial Sequence
  NA7S-H2-30 VHH
EVQLVESGGGLVQPGGSLRLSCAASGSFFRIVAMGWYRQAPGKGRELVATITRGGSSYYADSMKGRSTISRDNAKNTVYLQMNSLKPEDTAVYYCNVRVEVPFFQPNDYWGQGTLVTVSS

SEQ ID NO: 27 - protein, 123 aa, Artificial Sequence
  NA4S-H7-10 VHH
EVQLVESGGGLVQPGGSLRLSCAASGSIFSINVMGWYRQAPGKQRELVAGISTGGTTRYADSVKGRFTISRDNAKNTLYLQMNSLRAEDTAVYYCNADLATSYSWPVRYLEVWGQGTLVTVSS

SEQ ID NO: 28 - protein, 123 aa, Artificial Sequence
  NA4S-H7-3 VHH
EVQLVESGGGLVQPGGSLRLSCAASGSIFSINVMSWYRQAPGKQRELVAGISAGGTTRYADSVKGRFTISRDNAKNTLYLQMNSLRAEDTAVYYCNADLAEATSWPVRYLEVWGQGTLVTVSS

SEQ ID NO: 29 - protein, 122 aa, Artificial Sequence
  NA8S-H9-57 VHH
EVQLVESGGGLVQPGGSLRLSCAASGLIFSNYAVGWFRQAPGKGLEFVAAITWSGGSTNYADSVKGRFTISRDNAKNTLYLQMNSLRAEDTAVYYCAGGFFATSYSGNYGYWGQGTLVTVSS

SEQ ID NO: 30 - protein, 10 aa, Artificial Sequence
  CDR1
GSIFSINVMG

SEQ ID NO: 31 - protein, 9 aa, Artificial Sequence
  CDR2
GISTGGTTR

SEQ ID NO: 32 - protein, 15 aa, Artificial Sequence
  CDR3
DLATATSWPVRYLEV

SEQ ID NO: 33 - protein, 15 aa, Artificial Sequence
  CDR3
DLATSYSWPVRYLEV

SEQ ID NO: 34 - protein, 10 aa, Artificial Sequence
  CDR1
GSIFSINVMS

SEQ ID NO: 35 - protein, 9 aa, Artificial Sequence
  CDR2
GISAGGTTR

SEQ ID NO: 36 - protein, 15 aa, Artificial Sequence
  CDR3
DLAEATSWPVRYLEV

SEQ ID NO: 37 - protein, 10 aa, Artificial Sequence
  CDR1
GSFFRIVAMG

SEQ ID NO: 38 - protein, 9 aa, Artificial Sequence
  CDR2
TITRGGSTY

SEQ ID NO: 39 - protein, 12 aa, Artificial Sequence
  CDR3
RVEVPFMQPNDY

SEQ ID NO: 40 - protein, 10 aa, Artificial Sequence
  CDR1
GSFFRIVAME

SEQ ID NO: 41 - protein, 10 aa, Artificial Sequence
  CDR1
GSFFRIVMYG

SEQ ID NO: 42 - protein, 12 aa, Artificial Sequence
  CDR3
RVEVPFMAPNDY

SEQ ID NO: 43 - protein, 9 aa, Artificial Sequence
  CDR2
TITRGGSSY

SEQ ID NO: 44 - protein, 12 aa, Artificial Sequence
  CDR3
RVEVPFFQPNDY

SEQ ID NO: 45 - protein, 10 aa, Artificial Sequence
  CDR1
GRTFSNYAVG

SEQ ID NO: 46 - protein, 10 aa, Artificial Sequence
  CDR2
AITWSGGSTN

SEQ ID NO: 47 - protein, 13 aa, Artificial Sequence
  CDR3
GFFATSYSGNYGY

SEQ ID NO: 48 - protein, 10 aa, Artificial Sequence
  CDR1
GLIFSNYAVG